European Patent Specification EP 4 127 243 B1, published November 22, 2023. Title: Prediction of radiotherapy response for prostate cancer subject based on immune checkpoint genes. Applicant: Koninklijke Philips N.V. The sequence listing filed with the application follows.

SEQUENCE LISTING (22 sequences)

SEQ ID NO: 1 - DNA, 1976 bp, Homo sapiens
agagaccagcagaacggcatcccagccacgacggccactttgctctgtctgctctccgccacggccctgctctgttccctgggacacccccgcccccacctcctcaggctgcctgatctgcccagctttccagctttcctctggattccggcctctggtcatccctccccaccctctctccaaggccctctcctggtctcccttcttctagaaccccttcctccacctccctctctgcagaacttctcctttaccccccaccccccaccactgccccctttccttttctgacctccttttggagggctcagcgctgcccagaccataggagagatgtgggaggctcagttcctgggcttgctgtttctgcagccgctttgggtggctccagtgaagcctctccagccaggggctgaggtcccggtggtgtgggcccaggagggggctcctgcccagctcccctgcagccccacaatccccctccaggatctcagccttctgcgaagagcaggggtcacttggcagcatcagccagacagtggcccgcccgctgccgcccccggccatcccctggcccccggccctcacccggcggcgccctcctcctgggggcccaggccccgccgctacacggtgctgagcgtgggtcccggaggcctgcgcagcgggaggctgcccctgcagccccgcgtccagctggatgagcgcggccggcagcgcggggacttctcgctatggctgcgcccagcccggcgcgcggacgccggcgagtaccgcgccgcggtgcacctcagggaccgcgccctctcctgccgcctccgtctgcgcctgggccaggcctcgatgactgccagccccccaggatctctcagagcctccgactgggtcattttgaactgctccttcagccgccctgaccgcccagcctctgtgcattggttccggaaccggggccagggccgagtccctgtccgggagtccccccatcaccacttagcggaaagcttcctcttcctgccccaagtcagccccatggactctgggccctggggctgcatcctcacctacagagatggcttcaacgtctccatcatgtataacctcactgttctgggtctggagcccccaactcccttgacagtgtacgctggagcaggttccagggtggggctgccctgccgcctgcctgctggtgtggggacccggtctttcctcactgccaagtggactcctcctgggggaggccctgacctcctggtgactggagacaatggcgactttacccttcgactagaggatgtgagccaggcccaggctgggacctacacctgccatatccatctgcaggaacagcagctcaatgccactgtcacattggcaatcatcacagtgactcccaaatcctttgggtcacctggatccctggggaagctgctttgtgaggtgactccagtatctggacaagaacgctttgtgtggagctctctggacaccccatcccagaggagtttctcaggaccttggctggaggcacaggaggcccagctcctttcccagccttggcaatgccagctgtaccagggggagaggcttcttggagcagcagtgtacttcacagagctgtctagcccaggtgcccaacgctctgggagagccccaggtgccctcccagcaggccacctcctgctgtttctcatccttggtgtcctttctctgctccttttggtgactggagcctttggctttcacctttggagaagacagtggcgaccaagacgattttctgccttagagcaagggattcaccctccgcaggctcagagcaagatagaggagctggagcaagaaccggagccggagccggagccggaaccggagcccgagcccgagcccgagccggagcagctctgacctggagctgaggcagccagcagatctcagcagcccagtccaaataaactccctgtcagcagcaa

SEQ ID NO: 2 - protein, 525 aa, Homo sapiens
MWEAQFLGLLFLQPLWVAPVKPLQPGAEVPVVWAQEGAPAQLPCSPTIPLQDLSLLRRAGVTWQHQPDSGPPAAAPGHPLAPGPHPAAPSSWGPRPRRYTVLSVGPGGLRSGRLPLQPRVQLDERGRQRGDFSLWLRPARRADAGEYRAAVHLRDRALSCRLRLRLGQASMTASPPGSLRASDWVILNCSFSRPDRPASVHWFRNRGQGRVPVRESPHHHLAESFLFLPQVSPMDSGPWGCILTYRDGFNVSIMYNLTVLGLEPPTPLTVYAGAGSRVGLPCRLPAGVGTRSFLTAKWTPPGGGPDLLVTGDNGDFTLRLEDVSQAQAGTYTCHIHLQEQQLNATVTLAIITVTPKSFGSPGSLGKLLCEVTPVSGQERFVWSSLDTPSQRSFSGPWLEAQEAQLLSQPWQCQLYQGERLLGAAVYFTELSSPGAQRSGRAPGALPAGHLLLFLILGVLSLLLLVTGAFGFHLWRRQWRPRRFSALEQGIHPPQAQSKIEELEQEPEPEPEPEPEPEPEPEPEQL

SEQ ID NO: 3 - DNA, 1628 bp, Homo sapiens
ctttgttaagtcgttccctctacaaaggacttcctagtgggtgtgaaaggcagcggtggccacagaggcggcggagagatggccttcagcggttcccaggctccctacctgagtccagctgtccccttttctgggactattcaaggaggtctccaggacggacttcagatcactgtcaatgggaccgttctcagctccagtggaaccaggtttgctgtgaactttcagactggcttcagtggaaatgacattgccttccacttcaaccctcggtttgaagatggagggtacgtggtgtgcaacacgaggcagaacggaagctgggggcccgaggagaggaagacacacatgcctttccagaaggggatgccctttgacctctgcttcctggtgcagagctcagatttcaaggtgatggtgaacgggatcctcttcgtgcagtacttccaccgcgtgcccttccaccgtgtggacaccatctccgtcaatggctctgtgcagctgtcctacatcagcttccagcctcccggcgtgtggcctgccaacccggctcccattacccagacagtcatccacacagtgcagagcgcccctggacagatgttctctactcccgccatcccacctatgatgtacccccaccccgcctatccgatgcctttcatcaccaccattctgggagggctgtacccatccaagtccatcctcctgtcaggcactgtcctgcccagtgctcagaggttccacatcaacctgtgctctgggaaccacatcgccttccacctgaacccccgttttgatgagaatgctgtggtccgcaacacccagatcgacaactcctgggggtctgaggagcgaagtctgccccgaaaaatgcccttcgtccgtggccagagcttctcagtgtggatcttgtgtgaagctcactgcctcaaggtggccgtggatggtcagcacctgtttgaatactaccatcgcctgaggaacctgcccaccatcaacagactggaagtggggggcgacatccagctgacccatgtgcagacataggcggcttcctggccctggggccgggggctggggtgtggggcagtctgggtcctctcatcatccccacttcccaggcccagcctttccaaccctgcctgggatctgggctttaatgcagaggccatgtccttgtctggtcctgcttctggctacagccaccctggaacggagaaggcagctgacggggattgccttcctcagccgcagcagcacctggggctccagctgctggaatcctaccatcccaggaggcaggcacagccagggagaggggaggagtgggcagtgaagatgaagccccatgctcagtcccctcccatcccccacgcagctccaccccagtcccaagccaccagctgtctgctcctggtgggaggtggcctcctcagcccctcctctctgacctttaacctcactctcaccttgcaccgtgcaccaacccttcacccctcctggaaagcaggcctgatggcttcccactggcctccaccacctgaccagagtgttctcttcagaggactggctcctttcccagtgtccttaaaataaagaaatgaaaatgcttgttggcacattca

SEQ ID NO: 4 - DNA, 1724 bp, Homo sapiens
ctttgttaagtcgttccctctacaaaggacttcctagtgggtgtgaaaggcagcggtggccacagaggcggcggagagatggccttcagcggttcccaggctccctacctgagtccagctgtccccttttctgggactattcaaggaggtctccaggacggacttcagatcactgtcaatgggaccgttctcagctccagtggaaccaggtttgctgtgaactttcagactggcttcagtggaaatgacattgccttccacttcaaccctcggtttgaagatggagggtacgtggtgtgcaacacgaggcagaacggaagctgggggcccgaggagaggaagacacacatgcctttccagaaggggatgccctttgacctctgcttcctggtgcagagctcagatttcaaggtgatggtgaacgggatcctcttcgtgcagtacttccaccgcgtgcccttccaccgtgtggacaccatctccgtcaatggctctgtgcagctgtcctacatcagcttccagaacccccgcacagtccctgttcagcctgccttctccacggtgccgttctcccagcctgtctgtttcccacccaggcccagggggcgcagacaaaaacctcccggcgtgtggcctgccaacccggctcccattacccagacagtcatccacacagtgcagagcgcccctggacagatgttctctactcccgccatcccacctatgatgtacccccaccccgcctatccgatgcctttcatcaccaccattctgggagggctgtacccatccaagtccatcctcctgtcaggcactgtcctgcccagtgctcagaggttccacatcaacctgtgctctgggaaccacatcgccttccacctgaacccccgttttgatgagaatgctgtggtccgcaacacccagatcgacaactcctgggggtctgaggagcgaagtctgccccgaaaaatgcccttcgtccgtggccagagcttctcagtgtggatcttgtgtgaagctcactgcctcaaggtggccgtggatggtcagcacctgtttgaatactaccatcgcctgaggaacctgcccaccatcaacagactggaagtggggggcgacatccagctgacccatgtgcagacataggcggcttcctggccctggggccgggggctggggtgtggggcagtctgggtcctctcatcatccccacttcccaggcccagcctttccaaccctgcctgggatctgggctttaatgcagaggccatgtccttgtctggtcctgcttctggctacagccaccctggaacggagaaggcagctgacggggattgccttcctcagccgcagcagcacctggggctccagctgctggaatcctaccatcccaggaggcaggcacagccagggagaggggaggagtgggcagtgaagatgaagccccatgctcagtcccctcccatcccccacgcagctccaccccagtcccaagccaccagctgtctgctcctggtgggaggtggcctcctcagcccctcctctctgacctttaacctcactctcaccttgcaccgtgcaccaacccttcacccctcctggaaagcaggcctgatggcttcccactggcctccaccacctgaccagagtgttctcttcagaggactggctcctttcccagtgtccttaaaataaagaaatgaaaatgcttgttggcacattca

SEQ ID NO: 5 - DNA, 1465 bp, Homo sapiens
ctttgttaagtcgttccctctacaaaggacttcctagtgggtgtgaaaggcagcggtggccacagaggcggcggagagatggccttcagcggttcccaggctccctacctgagtccagctgtccccttttctgggactattcaaggaggtctccaggacggacttcagatcactgtcaatgggaccgttctcagctccagtggaaccaggtttgctgtgaactttcagactggcttcagtggaaatgacattgccttccacttcaaccctcggtttgaagatggagggtacgtggtgtgcaacacgaggcagaacggaagctgggggcccgaggagaggaagacacacatgcctttccagaaggggatgccctttgacctctgcttcctggtgcagagctcagatttcaaggtgatggtgaacgggatcctcttcgtgcagtacttccaccgcgtgcccttccaccgtgtggacaccatctccgtcaatggctctgtgcagctgtcctacatcagcttccagcctcccggcgtgtggcctgccaacccggctcccattacccagacagtcatccacacagtgcagagcgcccctggacagatgttctctactcccgccatcccacctatgatgtacccccaccccgcctatccgatgcctttcatcaccaccattctgggagggctgtacccatccaagtccatcctcctgtcaggcactgtcctgcccagtgctcagaggtgtggatcttgtgtgaagctcactgcctcaaggtggccgtggatggtcagcacctgtttgaatactaccatcgcctgaggaacctgcccaccatcaacagactggaagtggggggcgacatccagctgacccatgtgcagacataggcggcttcctggccctggggccgggggctggggtgtggggcagtctgggtcctctcatcatccccacttcccaggcccagcctttccaaccctgcctgggatctgggctttaatgcagaggccatgtccttgtctggtcctgcttctggctacagccaccctggaacggagaaggcagctgacggggattgccttcctcagccgcagcagcacctggggctccagctgctggaatcctaccatcccaggaggcaggcacagccagggagaggggaggagtgggcagtgaagatgaagccccatgctcagtcccctcccatcccccacgcagctccaccccagtcccaagccaccagctgtctgctcctggtgggaggtggcctcctcagcccctcctctctgacctttaacctcactctcaccttgcaccgtgcaccaacccttcacccctcctggaaagcaggcctgatggcttcccactggcctccaccacctgaccagagtgttctcttcagaggactggctcctttcccagtgtccttaaaataaagaaatgaaaatgcttgttggcacattca

SEQ ID NO: 6 - protein, 323 aa, Homo sapiens
MAFSGSQAPYLSPAVPFSGTIQGGLQDGLQITVNGTVLSSSGTRFAVNFQTGFSGNDIAFHFNPRFEDGGYVVCNTRQNGSWGPEERKTHMPFQKGMPFDLCFLVQSSDFKVMVNGILFVQYFHRVPFHRVDTISVNGSVQLSYISFQPPGVWPANPAPITQTVIHTVQSAPGQMFSTPAIPPMMYPHPAYPMPFITTILGGLYPSKSILLSGTVLPSAQRFHINLCSGNHIAFHLNPRFDENAVVRNTQIDNSWGSEERSLPRKMPFVRGQSFSVWILCEAHCLKVAVDGQHLFEYYHRLRNLPTINRLEVGGDIQLTHVQT

SEQ ID NO: 7 - protein, 355 aa, Homo sapiens
MAFSGSQAPYLSPAVPFSGTIQGGLQDGLQITVNGTVLSSSGTRFAVNFQTGFSGNDIAFHFNPRFEDGGYVVCNTRQNGSWGPEERKTHMPFQKGMPFDLCFLVQSSDFKVMVNGILFVQYFHRVPFHRVDTISVNGSVQLSYISFQNPRTVPVQPAFSTVPFSQPVCFPPRPRGRRQKPPGVWPANPAPITQTVIHTVQSAPGQMFSTPAIPPMMYPHPAYPMPFITTILGGLYPSKSILLSGTVLPSAQRFHINLCSGNHIAFHLNPRFDENAVVRNTQIDNSWGSEERSLPRKMPFVRGQSFSVWILCEAHCLKVAVDGQHLFEYYHRLRNLPTINRLEVGGDIQLTHVQT

SEQ ID NO: 8 - protein, 246 aa, Homo sapiens
MAFSGSQAPYLSPAVPFSGTIQGGLQDGLQITVNGTVLSSSGTRFAVNFQTGFSGNDIAFHFNPRFEDGGYVVCNTRQNGSWGPEERKTHMPFQKGMPFDLCFLVQSSDFKVMVNGILFVQYFHRVPFHRVDTISVNGSVQLSYISFQPPGVWPANPAPITQTVIHTVQSAPGQMFSTPAIPPMMYPHPAYPMPFITTILGGLYPSKSILLSGTVLPSAQRCGSCVKLTASRWPWMVSTCLNTTIA

SEQ ID NO: 9 - DNA, 1700 bp, Homo sapiens
aggtcaatgatagcatctgcctagagtcaaacctccgtgcttctcagacagtgccttttcaccatgagtgggtgcccatttttaggaaacaactttggatatacttttaaaaaactccccgtagaaggcagcgaagaagacaaatcacaaactggtgtgaatagagccagcaaaggaggtcttatctatgggaactacctgcatttggaaaaagttttgaatgcacaagaactgcaaagtgaaacaaaaggaaataaaatccatgatgaacatctttttatcataactcatcaagcttatgaactctggtttaagcaaatcctctgggagttggattctgttcgagagatctttcagaatggccatgtcagagatgaaaggaacatgcttaaggttgtttctcggatgcaccgagtgtcagtgatcctgaaactgctggtgcagcagttttccattctggagacgatgacagccttggacttcaatgacttcagagagtacttatctccagcatcaggcttccagagtttgcaattccgactattagaaaacaagataggtgttcttcagaacatgagagtcccttataacagaagacattatcgtgataacttcaaaggagaagaaaatgaactgctacttaaatctgagcaggaaaagacacttctggaattagtggaggcatggctggaaagaactccaggtttagagccacatggatttaacttctggggaaagcttgaaaaaaatatcaccagaggcctggaagaggaattcataaggattcaggctaaagaagagtctgaagaaaaagaggaacaggtggctgaatttcagaagcaaaaagaggtgctactgtccttatttgatgagaaacgtcatgaacatctccttagtaaaggtgaaagacggctgtcatacagagcacttcagggagcattgatgatatatttttacagggaagagcctaggttccaggtgccttttcagttgctgacttctcttatggacatagattcactgatgaccaaatggagatataaccatgtgtgcatggtgcacagaatgctgggcagcaaagctggcaccggtggttcctcaggctatcactacctgcgatcaactgtgagtgataggtacaaggtatttgtagatttatttaatctttcaacatacctgattccccgacactggataccgaagatgaacccaaccattcacaaatttctatatacagcagaatactgtgatagctcctacttcagcagtgatgaatcagattaaaatcgtctgcaaaatctatgaagaatactggtttcacagcctattttttattttctatggattttcataaatacagtttgaatatatgtatgcatatattgttcagcaccacgatgctctgatttaattctagaaacaatttgattacctcttgtttgtgacaagactaagcattaagatgagaaagaatacatttaaatagtaacattgtacatagggtgttttcctattaaaaattcagtttcccctgagacttaatgtaaccacttaatgtaatcactatctcattgtttcatctttataaacttgtaaacttcatctatttcaaatattttatgcagtacattatattattctgtacaaaggctttcaaacaaaatttttaaaataataaagtattaatctttctccctgta

SEQ ID NO: 10 - protein, 406 aa, Homo sapiens
MSGCPFLGNNFGYTFKKLPVEGSEEDKSQTGVNRASKGGLIYGNYLHLEKVLNAQELQSETKGNKIHDEHLFIITHQAYELWFKQILWELDSVREIFQNGHVRDERNMLKVVSRMHRVSVILKLLVQQFSILETMTALDFNDFREYLSPASGFQSLQFRLLENKIGVLQNMRVPYNRRHYRDNFKGEENELLLKSEQEKTLLELVEAWLERTPGLEPHGFNFWGKLEKNITRGLEEEFIRIQAKEESEEKEEQVAEFQKQKEVLLSLFDEKRHEHLLSKGERRLSYRALQGALMIYFYREEPRFQVPFQLLTSLMDIDSLMTKWRYNHVCMVHRMLGSKAGTGGSSGYHYLRSTVSDRYKVFVDLFNLSTYLIPRHWIPKMNPTIHKFLYTAEYCDSSYFSSDESD

SEQ ID NO: 11 - DNA, 1282 bp, Homo sapiens
ggaagtctgtcaactgggagggggagaggggggtgatgggccaggaatggggtccccgggcatggtgctgggcctcctggtgcagatctgggccctgcaagaagcctcaagcctgagcgtgcagcaggggcccaacttgctgcaggtgaggcagggcagtcaggcgaccctggtctgccaggtggaccaggccacagcctgggaacggctccgtgttaagtggacaaaggatggggccatcctgtgtcaaccgtacatcaccaacggcagcctcagcctgggggtctgcgggccccagggacggctctcctggcaggcacccagccatctcaccctgcagctggaccctgtgagcctcaaccacagcggggcgtacgtgtgctgggcggccgtagagattcctgagttggaggaggctgagggcaacataacaaggctctttgtggacccagatgaccccacacagaacagaaaccggatcgcaagcttcccaggattcctcttcgtgctgctgggggtgggaagcatgggtgtggctgcgatcgtgtggggtgcctggttctggggccgccgcagctgccagcaaagggactcaggtaacagcccaggaaatgcattctacagcaacgtcctataccggccccggggggccccaaagaagagtgaggactgctctggagaggggaaggaccagaggggccagagcatttattcaacctccttcccgcaaccggccccccgccagccgcacctggcgtcaagaccctgccccagcccgagaccctgccccagccccaggcccggccaccccgtctctatggtcagggtctctcctagaccaagccccacccagcagccgaggccaaaagggttccccaaagtgggagaggagtgagagatcccaggagacctcaacaggaccccacccataggtacacacaaaaaaggggggatcgaggccagacacggtggctcacgcctgtaatcccagcagtttgggaagccgaggcgggtggaacacttgaggtcaggggtttgagaccagcctggcttgaacctgggaggcggaggttgcagtgagccgagattgcgccactgcactccagcctgggcgacagagtgagactccgtctcaaaaaaaacaaaaagcaggaggattgggagcctgtcagccccatcctgagaccccgtcctcatttctgtaatgatggatctcgctcccactttcccccaagaacctaataaaggcttgtgaagaaaaagcaaaaaaaaaaaaaaaaaa

SEQ ID NO: 12 - DNA, 1270 bp, Homo sapiens
ggaagtctgtcaactgggagggggagaggggggtgatgggccaggaatggggtccccgggcatggtgctgggcctcctggtgcagatctgggccctgcaagaagcctcaagcctgagcgtgcagcaggggcccaacttgctgcaggtgaggcagggcagtcaggcgaccctggtctgccaggtggaccaggccacagcctgggaacggctccgtgttaagtggacaaaggatggggccatcctgtgtcaaccgtacatcaccaacggcagcctcagcctgggggtctgcgggccccagggacggctctcctggcaggcacccagccatctcaccctgcagctggaccctgtgagcctcaaccacagcggggcgtacgtgtgctgggcggccgtagagattcctgagttggaggaggctgagggcaacataacaaggctctttgtggacccagatgaccccacacagaacagaaaccggatcgcaagcttcccaggattcctcttcgtgctgctgggggtgggaagcatgggtgtggctgcgatcgtgtggggtgcctggttctggggccgccgcagctgccagcaaagggactcaggaaatgcattctacagcaacgtcctataccggccccggggggccccaaagaagagtgaggactgctctggagaggggaaggaccagaggggccagagcatttattcaacctccttcccgcaaccggccccccgccagccgcacctggcgtcaagaccctgccccagcccgagaccctgccccagccccaggcccggccaccccgtctctatggtcagggtctctcctagaccaagccccacccagcagccgaggccaaaagggttccccaaagtgggagaggagtgagagatcccaggagacctcaacaggaccccacccataggtacacacaaaaaaggggggatcgaggccagacacggtggctcacgcctgtaatcccagcagtttgggaagccgaggcgggtggaacacttgaggtcaggggtttgagaccagcctggcttgaacctgggaggcggaggttgcagtgagccgagattgcgccactgcactccagcctgggcgacagagtgagactccgtctcaaaaaaaacaaaaagcaggaggattgggagcctgtcagccccatcctgagaccccgtcctcatttctgtaatgatggatctcgctcccactttcccccaagaacctaataaaggcttgtgaagaaaaagcaaaaaaaaaaaaaaaaaa

SEQ ID NO: 13 - DNA, 918 bp, Homo sapiens
ggaagtctgtcaactgggagggggagaggggggtgatgggccaggaatggggtccccgggcatggtgctgggcctcctggtgcagatctgggatgaccccacacagaacagaaaccggatcgcaagcttcccaggattcctcttcgtgctgctgggggtgggaagcatgggtgtggctgcgatcgtgtggggtgcctggttctggggccgccgcagctgccagcaaagggactcaggtaacagcccaggaaatgcattctacagcaacgtcctataccggccccggggggccccaaagaagagtgaggactgctctggagaggggaaggaccagaggggccagagcatttattcaacctccttcccgcaaccggccccccgccagccgcacctggcgtcaagaccctgccccagcccgagaccctgccccagccccaggcccggccaccccgtctctatggtcagggtctctcctagaccaagccccacccagcagccgaggccaaaagggttccccaaagtgggagaggagtgagagatcccaggagacctcaacaggaccccacccataggtacacacaaaaaaggggggatcgaggccagacacggtggctcacgcctgtaatcccagcagtttgggaagccgaggcgggtggaacacttgaggtcaggggtttgagaccagcctggcttgaacctgggaggcggaggttgcagtgagccgagattgcgccactgcactccagcctgggcgacagagtgagactccgtctcaaaaaaaacaaaaagcaggaggattgggagcctgtcagccccatcctgagaccccgtcctcatttctgtaatgatggatctcgctcccactttcccccaagaacctaataaaggcttgtgaagaaaaagcaaaaaaaaaaaaaa

SEQ ID NO: 14 - protein, 282 aa, Homo sapiens
MGSPGMVLGLLVQIWALQEASSLSVQQGPNLLQVRQGSQATLVCQVDQATAWERLRVKWTKDGAILCQPYITNGSLSLGVCGPQGRLSWQAPSHLTLQLDPVSLNHSGAYVCWAAVEIPELEEAEGNITRLFVDPDDPTQNRNRIASFPGFLFVLLGVGSMGVAAIVWGAWFWGRRSCQQRDSGNSPGNAFYSNVLYRPRGAPKKSEDCSGEGKDQRGQSIYSTSFPQPAPRQPHLASRPCPSPRPCPSPRPGHPVSMVRVSPRPSPTQQPRPKGFPKVGEE

SEQ ID NO: 15 - protein, 278 aa, Homo sapiens
MGSPGMVLGLLVQIWALQEASSLSVQQGPNLLQVRQGSQATLVCQVDQATAWERLRVKWTKDGAILCQPYITNGSLSLGVCGPQGRLSWQAPSHLTLQLDPVSLNHSGAYVCWAAVEIPELEEAEGNITRLFVDPDDPTQNRNRIASFPGFLFVLLGVGSMGVAAIVWGAWFWGRRSCQQRDSGNAFYSNVLYRPRGAPKKSEDCSGEGKDQRGQSIYSTSFPQPAPRQPHLASRPCPSPRPCPSPRPGHPVSMVRVSPRPSPTQQPRPKGFPKVGEE

SEQ ID NO: 16 - protein, 162 aa, Homo sapiens
MGSPGMVLGLLVQIWDDPTQNRNRIASFPGFLFVLLGVGSMGVAAIVWGAWFWGRRSCQQRDSGNSPGNAFYSNVLYRPRGAPKKSEDCSGEGKDQRGQSIYSTSFPQPAPRQPHLASRPCPSPRPCPSPRPGHPVSMVRVSPRPSPTQQPRPKGFPKVGEE

SEQ ID NO: 17 - DNA, 2734 bp, Homo sapiens
ctggtaatctgtggcgtaacaagacctccaggtgattctctgtattagcagccgctctgtgctccctgattcctccagaaaagcacaaggatttaatccagatagatataaatttcacctgggatcatttatcattccacattcttctttaagaaatgtgctaaagagccacagatgggtcttgatgaaaacaaaggaaaagccatgaagtttctacagcataattagcatcatcattattctggctggagcaattgcactcatcattggctttggtatttcagggagacactccatcacagtcactactgtcgcctcagctgggaacattggggaggatggaatcctgagctgcacttttgaacctgacatcaaactttctgatatcgtgatacaatggctgaaggaaggtgttttaggcttggtccatgagttcaaagaaggcaaagatgagctgtcggagcaggatgaaatgttcagaggccggacagcagtgtttgctgatcaagtgatagttggcaatgcctctttgcggctgaaaaacgtgcaactcacagatgctggcacctacaaatgttatatcatcacttctaaaggcaaggggaatgctaaccttgagtataaaactggagccttcagcatgccggaagtgaatgtggactataatgccagctcagagaccttgcggtgtgaggctccccgatggttcccccagcccacagtggtctgggcatcccaagttgaccagggagccaacttctcggaagtctccaataccagctttgagctgaactctgagaatgtgaccatgaaggttgtgtctgtgctctacaatgttacgatcaacaacacatactcctgtatgattgaaaatgacattgccaaagcaacaggggatatcaaagtgacagaatcggagatcaaaaggcggagtcacctacagctgctaaactcaaaggcttctctgtgtgtctcttctttctttgccatcagctgggcacttctgcctctcagcccttacctgatgctaaaataatgtgcctcggccacaaaaaagcatgcaaagtcattgttacaacagggatctacagaactatttcaccaccagatatgacctagttttatatttctgggaggaaatgaattcatatctagaagtctggagtgagcaaacaagagcaagaaacaaaaagaagccaaaagcagaaggctccaatatgaacaagataaatctatcttcaaagacatattagaagttgggaaaataattcatgtgaactagacaagtgtgttaagagtgataagtaaaatgcacgtggagacaagtgcatccccagatctcagggacctccccctgcctgtcacctggggagtgagaggacaggatagtgcatgttctttgtctctgaatttttagttatatgtgctgtaatgttgctctgaggaagcccctggaaagtctatcccaacatatccacatcttatattccacaaattaagctgtagtatgtaccctaagacgctgctaattgactgccacttcgcaactcaggggcggctgcattttagtaatgggtcaaatgattcactttttatgatgcttccaaaggtgccttggcttctcttcccaactgacaaatgccaaagttgagaaaaatgatcataattttagcataaacagagcagtcggcgacaccgattttataaataaactgagcaccttctttttaaacaaacaaatgcgggtttatttctcagatgatgttcatccgtgaatggtccagggaaggacctttcaccttgtctatatggcattatgtcatcacaagctctgaggcttctcctttccatcctgcgtggacagctaagacctcagttttcaatagcatctagagcagtgggactcagctggggtgatttcgccccccatctccgggggaatgtctgaagacaattttggttacctcaatgagggagtggaggaggatacagtgctactaccaactagtggatagaggccagggatgctgctcaacctcctaccatgtacaggacgtctccccattacaactacccaatccgaagtgtcaactgtgtcagggctaagaaaccctggttttgagtagaaaagggcctggaaagaggggagccaacaaatctgtctgcttcctcacattagtcattggcaaataagcattctgtctctttggctgctgcctcagcacagagagccagaactctatcgggcaccaggataacatctctcagtgaacagagttgacaaggcctatgggaaatgcctgatgggattatcttcagcttgttgagcttctaagtttctttcccttcattctaccctgcaagccaagttctgtaagagaaatgcctgagttctagctcaggttttcttactctgaatttagatctccagaccctgcctggccacaattcaaattaaggcaacaaacatataccttccatgaagcacacacagacttttgaaagcaaggacaatgactgcttgaattgaggccttgaggaatgaagctttgaaggaaaagaatactttgtttccagcccccttcccacactcttcatgtgttaaccactgccttcctggaccttggagccacggtgactgtattacatgttgttatagaaaactgattttagagttctgatcgttcaagagaatgattaaatatacatttcctacaccaaaaaaaaaaaaaaa

SEQ ID NO: 18 - DNA, 2605 bp, Homo sapiens
gtgagtcaccaaggaaggcagcggcagctccactcagccagtacccagatacgctgggaaccttccccagccatggcttccctggggcagatcctcttctggagcataattagcatcatcattattctggctggagcaattgcactcatcattggctttggtatttcagggagacactccatcacagtcactactgtcgcctcagctgggaacattggggaggatggaatcctgagctgcacttttgaacctgacatcaaactttctgatatcgtgatacaatggctgaaggaaggtgttttaggcttggtccatgagttcaaagaaggcaaagatgagctgtcggagcaggatgaaatgttcagaggccggacagcagtgtttgctgatcaagtgatagttggcaatgcctctttgcggctgaaaaacgtgcaactcacagatgctggcacctacaaatgttatatcatcacttctaaaggcaaggggaatgctaaccttgagtataaaactggagccttcagcatgccggaagtgaatgtggactataatgccagctcagagaccttgcggtgtgaggctccccgatggttcccccagcccacagtggtctgggcatcccaagttgaccagggagccaacttctcggaagtctccaataccagctttgagctgaactctgagaatgtgaccatgaaggttgtgtctgtgctctacaatgttacgatcaacaacacatactcctgtatgattgaaaatgacattgccaaagcaacaggggatatcaaagtgacagaatcggagatcaaaaggcggagtcacctacagctgctaaactcaaaggcttctctgtgtgtctcttctttctttgccatcagctgggcacttctgcctctcagcccttacctgatgctaaaataatgtgcctcggccacaaaaaagcatgcaaagtcattgttacaacagggatctacagaactatttcaccaccagatatgacctagttttatatttctgggaggaaatgaattcatatctagaagtctggagtgagcaaacaagagcaagaaacaaaaagaagccaaaagcagaaggctccaatatgaacaagataaatctatcttcaaagacatattagaagttgggaaaataattcatgtgaactagacaagtgtgttaagagtgataagtaaaatgcacgtggagacaagtgcatccccagatctcagggacctccccctgcctgtcacctggggagtgagaggacaggatagtgcatgttctttgtctctgaatttttagttatatgtgctgtaatgttgctctgaggaagcccctggaaagtctatcccaacatatccacatcttatattccacaaattaagctgtagtatgtaccctaagacgctgctaattgactgccacttcgcaactcaggggcggctgcattttagtaatgggtcaaatgattcactttttatgatgcttccaaaggtgccttggcttctcttcccaactgacaaatgccaaagttgagaaaaatgatcataattttagcataaacagagcagtcggcgacaccgattttataaataaactgagcaccttctttttaaacaaacaaatgcgggtttatttctcagatgatgttcatccgtgaatggtccagggaaggacctttcaccttgtctatatggcattatgtcatcacaagctctgaggcttctcctttccatcctgcgtggacagctaagacctcagttttcaatagcatctagagcagtgggactcagctggggtgatttcgccccccatctccgggggaatgtctgaagacaattttggttacctcaatgagggagtggaggaggatacagtgctactaccaactagtggatagaggccagggatgctgctcaacctcctaccatgtacaggacgtctccccattacaactacccaatccgaagtgtcaactgtgtcagggctaagaaaccctggttttgagtagaaaagggcctggaaagaggggagccaacaaatctgtctgcttcctcacattagtcattggcaaataagcattctgtctctttggctgctgcctcagcacagagagccagaactctatcgggcaccaggataacatctctcagtgaacagagttgacaaggcctatgggaaatgcctgatgggattatcttcagcttgttgagcttctaagtttctttcccttcattctaccctgcaagccaagttctgtaagagaaatgcctgagttctagctcaggttttcttactctgaatttagatctccagaccctgcctggccacaattcaaattaaggcaacaaacatataccttccatgaagcacacacagacttttgaaagcaaggacaatgactgcttgaattgaggccttgaggaatgaagctttgaaggaaaagaatactttgtttccagcccccttcccacactcttcatgtgttaaccactgccttcctggaccttggagccacggtgactgtattacatgttgttatagaaaactgattttagagttctgatcgttcaagagaatgattaaatatacatttcctacacca

SEQ ID NO: 19 - DNA, 2304 bp, Homo sapiens
acactatttaaggccaatacacgggagctggttgtgagtcaccaaggaaggcagcggcagctccactcagccagtacccagatacgctgggaaccttccccagccatggcttccctggggcagatcctcttctggagcataattagcatcatcattattctggctggagcaattgcactcatcattggctttggtatttcagccttcagcatgccggaagtgaatgtggactataatgccagctcagagaccttgcggtgtgaggctccccgatggttcccccagcccacagtggtctgggcatcccaagttgaccagggagccaacttctcggaagtctccaataccagctttgagctgaactctgagaatgtgaccatgaaggttgtgtctgtgctctacaatgttacgatcaacaacacatactcctgtatgattgaaaatgacattgccaaagcaacaggggatatcaaagtgacagaatcggagatcaaaaggcggagtcacctacagctgctaaactcaaaggcttctctgtgtgtctcttctttctttgccatcagctgggcacttctgcctctcagcccttacctgatgctaaaataatgtgcctcggccacaaaaaagcatgcaaagtcattgttacaacagggatctacagaactatttcaccaccagatatgacctagttttatatttctgggaggaaatgaattcatatctagaagtctggagtgagcaaacaagagcaagaaacaaaaagaagccaaaagcagaaggctccaatatgaacaagataaatctatcttcaaagacatattagaagttgggaaaataattcatgtgaactagacaagtgtgttaagagtgataagtaaaatgcacgtggagacaagtgcatccccagatctcagggacctccccctgcctgtcacctggggagtgagaggacaggatagtgcatgttctttgtctctgaatttttagttatatgtgctgtaatgttgctctgaggaagcccctggaaagtctatcccaacatatccacatcttatattccacaaattaagctgtagtatgtaccctaagacgctgctaattgactgccacttcgcaactcaggggcggctgcattttagtaatgggtcaaatgattcactttttatgatgcttccaaaggtgccttggcttctcttcccaactgacaaatgccaaagttgagaaaaatgatcataattttagcataaacagagcagtcggcgacaccgattttataaataaactgagcaccttctttttaaacaaacaaatgcgggtttatttctcagatgatgttcatccgtgaatggtccagggaaggacctttcaccttgtctatatggcattatgtcatcacaagctctgaggcttctcctttccatcctgcgtggacagctaagacctcagttttcaatagcatctagagcagtgggactcagctggggtgatttcgccccccatctccgggggaatgtctgaagacaattttggttacctcaatgagggagtggaggaggatacagtgctactaccaactagtggatagaggccagggatgctgctcaacctcctaccatgtacaggacgtctccccattacaactacccaatccgaagtgtcaactgtgtcagggctaagaaaccctggttttgagtagaaaagggcctggaaagaggggagccaacaaatctgtctgcttcctcacattagtcattggcaaataagcattctgtctctttggctgctgcctcagcacagagagccagaactctatcgggcaccaggataacatctctcagtgaacagagttgacaaggcctatgggaaatgcctgatgggattatcttcagcttgttgagcttctaagtttctttcccttcattctaccctgcaagccaagttctgtaagagaaatgcctgagttctagctcaggttttcttactctgaatttagatctccagaccctgcctggccacaattcaaattaaggcaacaaacatataccttccatgaagcacacacagacttttgaaagcaaggacaatgactgcttgaattgaggccttgaggaatgaagctttgaaggaaaagaatactttgtttccagcccccttcccacactcttcatgtgttaaccactgccttcctggaccttggagccacggtgactgtattacatgttgttatagaaaactgattttagagttctgatcgttcaagagaatgattaaatatacatttcctacaccaaaaaaaaaaaaaaa

SEQ ID NO: 20 - protein, 187 aa, Homo sapiens
MFRGRTAVFADQVIVGNASLRLKNVQLTDAGTYKCYIITSKGKGNANLEYKTGAFSMPEVNVDYNASSETLRCEAPRWFPQPTVVWASQVDQGANFSEVSNTSFELNSENVTMKVVSVLYNVTINNTYSCMIENDIAKATGDIKVTESEIKRRSHLQLLNSKASLCVSSFFAISWALLPLSPYLMLK

SEQ ID NO: 21 - protein, 282 aa, Homo sapiens
MASLGQILFWSIISIIIILAGAIALIIGFGISGRHSITVTTVASAGNIGEDGILSCTFEPDIKLSDIVIQWLKEGVLGLVHEFKEGKDELSEQDEMFRGRTAVFADQVIVGNASLRLKNVQLTDAGTYKCYIITSKGKGNANLEYKTGAFSMPEVNVDYNASSETLRCEAPRWFPQPTVVWASQVDQGANFSEVSNTSFELNSENVTMKVVSVLYNVTINNTYSCMIENDIAKATGDIKVTESEIKRRSHLQLLNSKASLCVSSFFAISWALLPLSPYLMLK

SEQ ID NO: 22 - protein, 166 aa, Homo sapiens
MASLGQILFWSIISIIIILAGAIALIIGFGISAFSMPEVNVDYNASSETLRCEAPRWFPQPTVVWASQVDQGANFSEVSNTSFELNSENVTMKVVSVLYNVTINNTYSCMIENDIAKATGDIKVTESEIKRRSHLQLLNSKASLCVSSFFAISWALLPLSPYLMLK